European Patent Application EP 4 685 242 A1, published January 28, 2026. Title: Method for obtaining useful data for the prediction of a subject's response to Platelet Rich Plasma treatment. Applicant: Baigene, S.L. Application ES. The sequence listing filed with the application follows.

SEQUENCE LISTING (28 sequences)

SEQ ID NO: 1 - DNA, 18 bp, synthetic construct
  source 1..18: mol_type = other DNA
acagtgaacgaggccgca

SEQ ID NO: 2 - DNA, 25 bp, synthetic construct
  source 1..25: mol_type = other DNA
gacaattgaactccttcatcacaga

SEQ ID NO: 3 - DNA, 25 bp, synthetic construct
  source 1..25: mol_type = other DNA
agcttcgttgagaaactcaatcctt

SEQ ID NO: 4 - DNA, 24 bp, synthetic construct
  source 1..24: mol_type = other DNA
gcttcgttgagaaactcaatcctc

SEQ ID NO: 5 - DNA, 27 bp, synthetic construct
  source 1..27: mol_type = other DNA
tgcgctgttatctctttcttatagcca

SEQ ID NO: 6 - DNA, 23 bp, synthetic construct
  source 1..23: mol_type = other DNA
ctccacacttctccattcttcac

SEQ ID NO: 7 - DNA, 21 bp, synthetic construct
  source 1..21: mol_type = other DNA
gggtttgtcactgagacagca

SEQ ID NO: 8 - DNA, 21 bp, synthetic construct
  source 1..21: mol_type = other DNA
gggtttgtcactgagacagct

SEQ ID NO: 9 - DNA, 17 bp, synthetic construct
  source 1..17: mol_type = other DNA
gaagccatgcgccggac

SEQ ID NO: 10 - DNA, 16 bp, synthetic construct
  source 1..16: mol_type = other DNA
gacgatgcccatgccc

SEQ ID NO: 11 - DNA, 19 bp, synthetic construct
  source 1..19: mol_type = other DNA
cccacacctcgtccctttg

SEQ ID NO: 12 - DNA, 19 bp, synthetic construct
  source 1..19: mol_type = other DNA
cccacacctcgtccctttc

SEQ ID NO: 13 - DNA, 21 bp, synthetic construct
  source 1..21: mol_type = other DNA
tgagttctcttgggtcagggc

SEQ ID NO: 14 - DNA, 20 bp, synthetic construct
  source 1..20: mol_type = other DNA
cccactgactttgagagctg

SEQ ID NO: 15 - DNA, 21 bp, synthetic construct
  source 1..21: mol_type = other DNA
tgctgccctctttttagcagt

SEQ ID NO: 16 - DNA, 21 bp, synthetic construct
  source 1..21: mol_type = other DNA
tgctgccctctttttagcaga

SEQ ID NO: 17 - DNA, 22 bp, synthetic construct
  source 1..22: mol_type = other DNA
ctgtgctttctcgtcttcagca

SEQ ID NO: 18 - DNA, 17 bp, synthetic construct
  source 1..17: mol_type = other DNA
ggctgtgcttctgcctg

SEQ ID NO: 19 - DNA, 20 bp, synthetic construct
  source 1..20: mol_type = other DNA
ggagcccagataccccaaag

SEQ ID NO: 20 - DNA, 20 bp, synthetic construct
  source 1..20: mol_type = other DNA
ggagcccagataccccaaaa

SEQ ID NO: 21 - DNA, 21 bp, synthetic construct
  source 1..21: mol_type = other DNA
ggtcagaatggtgcccatcac

SEQ ID NO: 22 - DNA, 22 bp, synthetic construct
  source 1..22: mol_type = other DNA
cagatccaaggagaaagtcagg

SEQ ID NO: 23 - DNA, 16 bp, synthetic construct
  source 1..16: mol_type = other DNA
cagtgcgcgctacagc

SEQ ID NO: 24 - DNA, 17 bp, synthetic construct
  source 1..17: mol_type = other DNA
ccagtgcgcgctacagt

SEQ ID NO: 25 - DNA, 19 bp, synthetic construct
  source 1..19: mol_type = other DNA
gggtccctttgtcacggct

SEQ ID NO: 26 - DNA, 40 bp, synthetic construct
  source 1..40: mol_type = other DNA
acttattctgttagaaatatctagaaaactactacgacct

SEQ ID NO: 27 - DNA, 30 bp, synthetic construct
  source 1..30: mol_type = other DNA
tctcctaacaaactgtttcacatctttttt

SEQ ID NO: 28 - DNA, 30 bp, synthetic construct
  source 1..30: mol_type = other DNA
tctcctaacaaactgtttcacatctttttc